European Patent Specification EP 3 400 955 B1, published August 13, 2025. Title: Use of Cryptonin in Treatment of Breast Cancer. Applicant: ISTANBUL UNIVERSITESI. Application TR 2016/20086. The sequence listing filed with the application follows.

SEQUENCE LISTING (1 sequence)

SEQ ID NO: 1 - protein, 23 aa, Cryptotympana dubia
GLLNGLALRLGKRALKKIIKRLC